European Patent Application EP 4 180 810 A1, published May 17, 2023. Title: Fluorescent cross-linked RNase H mutant conjugate, miRNA combination and application thereof. Applicant: Shanghai Miran Biotech Co. Ltd. The sequence listing filed with the application follows.

SEQUENCE LISTING (37 sequences)

SEQ ID NO: 1 - DNA, 28 bp, Artificial Sequence
  P3-let7a
  misc_feature (28)..(28): 3' NH2-C6
aactatacaacctactacctcatttttt

SEQ ID NO: 2 - DNA, 28 bp, Artificial Sequence
  P5-let7a
  misc_feature (28)..(28): 5' NH2-C6
ttttttaactatacaacctactacctca

SEQ ID NO: 3 - DNA, 28 bp, Artificial Sequence
  P3-LNA-let7a
  misc_feature (28)..(28): 3' NH2-C6
aactatacaacctactacctcatttttt

SEQ ID NO: 4 - DNA, 27 bp, Artificial Sequence
  P3-1a
  misc_feature (27)..(27): 3' NH2-C6
ggagtctccaaagccacgtactttttt

SEQ ID NO: 5 - DNA, 28 bp, Artificial Sequence
  P-let7b
  misc_feature (28)..(28): 3' NH2-C6
aaccacacaacctactacctcatttttt

SEQ ID NO: 6 - DNA, 28 bp, Artificial Sequence
  P-m141
  misc_feature (28)..(28): 3' NH2-C6
ccatctttaccagacagtgttatttttt

SEQ ID NO: 7 - DNA, 29 bp, Artificial Sequence
  P-m155
  misc_feature (29)..(29): 3' NH2-C6
acccctatcacgattagcattaatttttt

SEQ ID NO: 8 - DNA, 28 bp, Artificial Sequence
  P-m375
  misc_feature (28)..(28): 3' NH2-C6
tcacgcgagccgaacgaacaaatttttt

SEQ ID NO: 9 - DNA, 30 bp, Artificial Sequence
  P-RNU6
  misc_feature (30)..(30): 3' NH2-C6
ccaattttagtatatgtgctgccgtttttt

SEQ ID NO: 10 - DNA, 28 bp, Artificial Sequence
  P-m34a
  misc_feature (28)..(28): 3' NH2-C6
acaaccagctaagacactgccatttttt

SEQ ID NO: 11 - DNA, 28 bp, Artificial Sequence
  P-m16
  misc_feature (28)..(28): 3' NH2-C6
cgccaatatttacgtgctgctatttttt

SEQ ID NO: 12 - DNA, 27 bp, Artificial Sequence
  P-m151
  misc_feature (27)..(27): 3' NH2-C6
cctcaaggagcttcagtctagtttttt

SEQ ID NO: 13 - DNA, 29 bp, Artificial Sequence
  P-m145
  misc_feature (29)..(29): 3' NH2-C6
agggattcctgggaaaactggactttttt

SEQ ID NO: 14 - RNA, 22 nt, Artificial Sequence
  let-7a
ugagguaguagguuguauaguu

SEQ ID NO: 15 - RNA, 23 nt, Artificial Sequence
  m155
uuaaugcuaaucgugauaggggu

SEQ ID NO: 16 - RNA, 22 nt, Artificial Sequence
  m141
uaacacugucugguaaagaugg

SEQ ID NO: 17 - DNA, 25 bp, Artificial Sequence
  Rp
ggaagacaatcttcatctccttctg

SEQ ID NO: 18 - DNA, 149 bp, Artificial Sequence
  RCA-1a
aagattgtgttgggaaggatggatggatgtttaagatgttgaggtgggtgtgataagaggtggtggagggagtgtggaaagggaggtaggttagtttttttggatggatggttgtaataggagtgagtatagggagagagaaggagatg

SEQ ID NO: 19 - RNA, 64 nt, Artificial Sequence
  1a
guacguggcuuuggagacuccguggaggaggucuuaucagaggcacgucaacaucuuaaagaug

SEQ ID NO: 20 - protein, 155 aa, Artificial Sequence
  E48Q
MLKQVEIFTDGSCLGNPGPGGYGAILRYRGREKTFSAGYTRTTNNRMQLMAAIVALEALKEHCEVILSTDSQYVRQGITQWIHNWKKRGWKTADKKPVKNVDLWQRLDAALGQHQIKWEWVKGHAGHPENERCDELARAAAMNPTLEDTGYQVEV

SEQ ID NO: 21 - DNA, 29 bp, Artificial Sequence
  P-m574-5p
  misc_feature (29)..(29): 3' NH2-C6
acacactcacacacacacactcatttttt

SEQ ID NO: 22 - DNA, 28 bp, Artificial Sequence
  P-m15b
  misc_feature (28)..(28): 3' NH2-C6
tgtaaaccatgatgtgctgctatttttt

SEQ ID NO: 23 - DNA, 28 bp, Artificial Sequence
  P-m125b
  misc_feature (28)..(28): 3' NH2-C6
tcacaagttagggtctcagggatttttt

SEQ ID NO: 24 - DNA, 28 bp, Artificial Sequence
  P-m193b
  misc_feature (28)..(28): 3' NH2-C6
agcgggactttgagggccagtttttttt

SEQ ID NO: 25 - DNA, 28 bp, Artificial Sequence
  P-m206
  misc_feature (28)..(28): 3' NH2-C6
ccacacacttccttacattccatttttt

SEQ ID NO: 26 - DNA, 28 bp, Artificial Sequence
  P-m486
  misc_feature (28)..(28): 3' NH2-C6
ctcggggcagctcagtacaggatttttt

SEQ ID NO: 27 - DNA, 28 bp, Artificial Sequence
  P-m429
  misc_feature (28)..(28): 3' NH2-C6
acggttttaccagacagtattatttttt

SEQ ID NO: 28 - DNA, 28 bp, Artificial Sequence
  P-m365
  misc_feature (28)..(28): 3' NH2-C6
ataaggatttttaggggcattatttttt

SEQ ID NO: 29 - DNA, 31 bp, Artificial Sequence
  P-m203a
  misc_feature (31)..(31): 3' NH2-C6
aactgttgaactgttaagaaccacttttttt

SEQ ID NO: 30 - DNA, 29 bp, Artificial Sequence
  P-m454
  misc_feature (29)..(29): 3' NH2-C6
accctataagcaatattgcactatttttt

SEQ ID NO: 31 - DNA, 28 bp, Artificial Sequence
  P-m1285
  misc_feature (28)..(28): 3' NH2-C6
aggtctcactttgttgcccagatttttt

SEQ ID NO: 32 - DNA, 28 bp, Artificial Sequence
  P-m126
  misc_feature (28)..(28): 3' NH2-C6
cgcattattactcacggtacgatttttt

SEQ ID NO: 33 - DNA, 28 bp, Artificial Sequence
  P-m21
  misc_feature (28)..(28): 3' NH2-C6
tcaacatcagtctgataagctatttttt

SEQ ID NO: 34 - DNA, 29 bp, Artificial Sequence
  P-m19a
  misc_feature (29)..(29): 3' NH2-C6
tcagttttgcatagatttgcacatttttt

SEQ ID NO: 35 - DNA, 28 bp, Artificial Sequence
  P-m200b
  misc_feature (28)..(28): 3' NH2-C6
tcatcattaccaggcagtattatttttt

SEQ ID NO: 36 - DNA, 28 bp, Artificial Sequence
  P-m181a-2*
  misc_feature (28)..(28): 3' NH2-C6
ggtacagtcaacggtcagtggttttttt

SEQ ID NO: 37 - DNA, 29 bp, Artificial Sequence
  P3-m191
  misc_feature (29)..(29): 3' NH2-C6
cagctgcttttgggattccgttgtttttt